European Patent Specification EP 3 652 326 B1, published October 9, 2024. Title: Means and methods for AAV gene therapy in humans. Applicant: uniQure IP B.V. The sequence listing filed with the application follows.

SEQUENCE LISTING (3 sequences)

SEQ ID NO: 1 - protein, 724 aa, adeno-associated virus 5
MSFVDHPPDWLEEVGEGLREFLGLEAGPPKPKPNQQHQDQARGLVLPGYNYLGPGNGLDRGEPVNRADEVAREHDISYNEQLEAGDNPYLKYNHADAEFQEKLADDTSFGGNLGKAVFQAKKRVLEPFGLVEEGAKTAPTGKRIDDHFPKRKKARTEEDSKPSTSSDAEAGPSGSQQLQIPAQPASSLGADTMSAGGGGPLGDNNQGADGVGNASGDWHCDSTWMGDRVVTKSTRTWVLPSYNNHQYREIKSGSVDGSNANAYFGYSTPWGYFDFNRFHSHWSPRDWQRLINNYWGFRPRSLRVKIFNIQVKEVTVQDSTTTIANNLTSTVQVFTDDDYQLPYVVGNGTEGCLPAFPPQVFTLPQYGYATLNRDNTENPTERSSFFCLEYFPSKMLRTGNNFEFTYNFEEVPFHSSFAPSQNLFKLANPLVDQYLYRFVSTNNTGGVQFNKNLAGRYANTYKNWFPGPMGRTQGWNLGSGVNRASVSAFATTNRMELEGASYQVPPQPNGMTNNLQGSNTYALENTMIFNSQPANPGTTATYLEGNMLITSESETQPVNRVAYNVGGQMATNNQSSTTAPATGTYNLQEIVPGSVWMERDVYLQGPIWAKIPETGAHFHPSPAMGGFGLKHPPPMMLIKNTPVPGNITSFSDVPVSSFITQYSTGQVTVEMEWELKKENSKRWNPEIQYTNNYNDPQFVDFAPDSTGEYRTTRPIGTRYLTRPL

SEQ ID NO: 2 - protein, 725 aa, Artificial Sequence
  AAV2 / AAV5 VP1 hybrid
MAADGYLPDWLEDTLSEGIRQWWKLKPGPPPPKPAERHKDDSRGLVLPGYKYLGPFNGLDKGEPVNEADAAALEHDKAYDRQLDSGDNPYLKYNHADAEFQERLKEDTSFGGNLGRAVFQAKKRVLEPLGLVEEPVKTAPTGKRIDDHFPKRKKARTEEDSKPSTSSDAEAGPSGSQQLQIPAQPASSLGADTMSAGGGGPLGDNNQGADGVGNASGDWHCDSTWMGDRVVTKSTRTWVLPSYNNHQYREIKSGSVDGSNANAYFGYSTPWGYFDFNRFHSHWSPRDWQRLINNYWGFRPRSLRVKIFNIQVKEVTVQDSTTTIANNLTSTVQVFTDDDYQLPYVVGNGTEGCLPAFPPQVFTLPQYGYATLNRDNTENPTERSSFFCLEYFPSKMLRTGNNFEFTYNFEEVPFHSSFAPSQNLFKLANPLVDQYLYRFVSTNNTGGVQFNKNLAGRYANTYKNWFPGPMGRTQGWNLGSGVNRASVSAFATTNRMELEGASYQVPPQPNGMTNNLQGSNTYALENTMIFNSQPANPGTTATYLEGNMLITSESETQPVNRVAYNVGGQMATNNQSSTTAPATGTYNLQEIVPGSVWMERDVYLQGPIWAKIPETGAHFHPSPAMGGFGLKHPPPMMLIKNTPVPGNITSFSDVPVSSFITQYSTGQVTVEMEWELKKENSKRWNPEIQYTNNYNDPQFVDFAPDSTGEYRTTRPIGTRYLTRPL

SEQ ID NO: 3 - protein, 725 aa, Artificial Sequence
  AAV5 - insertion of ala between AA1 and AA2
  misc_feature (2)..(2): ala insertion
MASFVDHPPDWLEEVGEGLREFLGLEAGPPKPKPNQQHQDQARGLVLPGYNYLGPGNGLDRGEPVNRADEVAREHDISYNEQLEAGDNPYLKYNHADAEFQEKLADDTSFGGNLGKAVFQAKKRVLEPFGLVEEGAKTAPTGKRIDDHFPKRKKARTEEDSKPSTSSDAEAGPSGSQQLQIPAQPASSLGADTMSAGGGGPLGDNNQGADGVGNASGDWHCDSTWMGDRVVTKSTRTWVLPSYNNHQYREIKSGSVDGSNANAYFGYSTPWGYFDFNRFHSHWSPRDWQRLINNYWGFRPRSLRVKIFNIQVKEVTVQDSTTTIANNLTSTVQVFTDDDYQLPYVVGNGTEGCLPAFPPQVFTLPQYGYATLNRDNTENPTERSSFFCLEYFPSKMLRTGNNFEFTYNFEEVPFHSSFAPSQNLFKLANPLVDQYLYRFVSTNNTGGVQFNKNLAGRYANTYKNWFPGPMGRTQGWNLGSGVNRASVSAFATTNRMELEGASYQVPPQPNGMTNNLQGSNTYALENTMIFNSQPANPGTTATYLEGNMLITSESETQPVNRVAYNVGGQMATNNQSSTTAPATGTYNLQEIVPGSVWMERDVYLQGPIWAKIPETGAHFHPSPAMGGFGLKHPPPMMLIKNTPVPGNITSFSDVPVSSFITQYSTGQVTVEMEWELKKENSKRWNPEIQYTNNYNDPQFVDFAPDSTGEYRTTRPIGTRYLTRPL